European Patent Specification EP 3 345 999 B1, published October 18, 2023. Title: Method for Preparing Induced Pluripotent Stem Cells Using Synthetic Peptide. Applicant: SEOUL NATIONAL UNIVERSITY R&DB FOUNDATION NANO INTELLIGENT BIOMEDICAL RNGINEERING CORPORATION CO. LTD. The sequence listing filed with the application follows.

SEQUENCE LISTING (5 sequences)

SEQ ID NO: 1 - protein, 15 aa, Artificial Sequence
  P1
GKCSTRGRKCCRRKK

SEQ ID NO: 2 - protein, 15 aa, Artificial Sequence
  P2
GKCSTRGRKCMRRKK

SEQ ID NO: 3 - protein, 15 aa, Artificial Sequence
  P3
GKCSTRGRKMCRRKK

SEQ ID NO: 4 - protein, 11 aa, Artificial Sequence
  C1
HRRCNKNNKKR

SEQ ID NO: 5 - protein, 19 aa, Artificial Sequence
  C2
GLRSKSKKFRRPDIQYPDA